European Patent Specification EP 3 801 771 B1, published October 23, 2024. Title: ANTIBODY COMPLEX AND USES THEREOF. Applicant: Diatheva srl. The sequence listing filed with the application follows.

SEQUENCE LISTING (42 sequences)

SEQ ID NO: 1 - protein, 9 aa, Artificial Sequence
  Amino acid sequence of CDR3 of the VH chain
AKSHKRFDY

SEQ ID NO: 2 - protein, 11 aa, Artificial Sequence
  Amino acid sequence of CDR3 of the VL chain
NSSFPRTSSVV

SEQ ID NO: 3 - protein, 10 aa, Artificial Sequence
  Amino acid sequence of CDR1 of the VH chain
GFTFSSYAMS

SEQ ID NO: 4 - protein, 9 aa, Artificial Sequence
  mino acid sequence of CDR2 of the VH chain
AISGSGGST

SEQ ID NO: 5 - protein, 11 aa, Artificial Sequence
  mino acid sequence of CDR1 of the VL chain
QGDSLRSYYAS

SEQ ID NO: 6 - protein, 7 aa, Artificial Sequence
  mino acid sequence of CDR2 of the VL chain
GKNNRPS

SEQ ID NO: 7 - protein, 116 aa, Artificial Sequence
  Amino acid sequence of the VH chain
EVQLVESGGGLVRPGGSLRLSCAASGFTFSSYAMSWVRQAPGKGLEWVSAISGSGGSTYYADSVKGRFTISRDNSKNTLYLQMNSLRAEDTAVYYCAKSHKRFDYWGQGTLVTVSR

SEQ ID NO: 8 - protein, 109 aa, Artificial Sequence
  Amino acid sequence of the VL chain
SSELTQDPAVSVALGQTVRITCQGDSLRSYYASWYQQKPGQAPVLVIYGKNNRPSGIPDRFSGSSSGNTASLTITGAQAEDEADYYCNSSFPRTSSVVFGGGTKLTVLG

SEQ ID NO: 9 - protein, 5 aa, Artificial Sequence
  Amino acid sequence of the linker component unit
GGGGS

SEQ ID NO: 10 - protein, 229 aa, Artificial Sequence
  Amino acid sequence of the scFv unit of the scFv multivalent molecule
EVQLVESGGGLVRPGGSLRLSCAASGFTFSSYAMSWVRQAPGKGLEWVSAISGSGGSTYYADSVKGRFTISRDNSKNTLYLQMNSLRAEDTAVYYCAKSHKRFDYWGQGTLVTVSRGGGGSSELTQDPAVSVALGQTVRITCQGDSLRSYYASWYQQKPGQAPVLVIYGKNNRPSGIPDRFSGSSSGNTASLTITGAQAEDEADYYCNSSFPRTSSVVFGGGTKLTVLG

SEQ ID NO: 11 - DNA, 27 bp, Artificial Sequence
  Nucleotide sequence of the CDR3 of the VH chain
gcgaaatcgcataagcgttttgactac

SEQ ID NO: 12 - DNA, 33 bp, Artificial Sequence
  Nucleotide sequence of the CDR3 of the VL chain
aactcctcttttccccggacttcttctgtggta

SEQ ID NO: 13 - DNA, 30 bp, Artificial Sequence
  Nucleotide sequence of the CDR1 of the VH chain
ggattcacctttagcagctatgccatgagc

SEQ ID NO: 14 - DNA, 27 bp, Artificial Sequence
  Nucleotide sequence of the CDR2 of the VH chain
gctattagtggtagtggtggtagcaca

SEQ ID NO: 15 - DNA, 33 bp, Artificial Sequence
  Nucleotide sequence of the CDR1 of the VL chain
caaggagacagcctcagaagctattatgcaagc

SEQ ID NO: 16 - DNA, 21 bp, Artificial Sequence
  Nucleotide sequence of the CDR2 of the VL chain
ggtaaaaacaaccggccctca

SEQ ID NO: 17 - DNA, 348 bp, Artificial Sequence
  Nucleotide sequence of the VH chain
gaggtgcagctggtggagtctgggggaggcttggtacggcctggggggtccctgagactctcctgtgcagcctctggattcacctttagcagctatgccatgagctgggtccgccaggctccagggaaggggctggagtgggtctcagctattagtggtagtggtggtagcacatactacgcagactccgtgaagggccggttcaccatctccagagacaattccaagaacacgctgtatctgcaaatgaacagcctgagagccgaggacacggccgtatattactgtgcgaaatcgcataagcgttttgactactggggccagggaaccctggtcaccgtgtcgaga

SEQ ID NO: 18 - DNA, 327 bp, Artificial Sequence
  Nucleotide sequence of the VL chain
tgctctgagctgactcaggaccctgctgtgtctgtggccttgggacagacagtcaggatcacatgccaaggagacagcctcagaagctattatgcaagctggtaccagcagaagccaggacaggcccctgtacttgtcatctatggtaaaaacaaccggccctcagggatcccagaccgattctctggctccagctcaggaaacacagcttccttgaccatcactggggctcaggcggaagatgaggctgactattactgtaactcctcttttccccggacttcttctgtggtattcggcggagggaccaagctgaccgtcctaggc

SEQ ID NO: 19 - DNA, 15 bp, Artificial Sequence
  Nucleotide sequence of the component of the linker
ggcggtggcggatcg

SEQ ID NO: 20 - DNA, 687 bp, Artificial Sequence
  Nucleotide sequence of the scFv unit of the scFv multivalent molecule
gaggtgcagctggtggagtctgggggaggcttggtacggcctggggggtccctgagactctcctgtgcagcctctggattcacctttagcagctatgccatgagctgggtccgccaggctccagggaaggggctggagtgggtctcagctattagtggtagtggtggtagcacatactacgcagactccgtgaagggccggttcaccatctccagagacaattccaagaacacgctgtatctgcaaatgaacagcctgagagccgaggacacggccgtatattactgtgcgaaatcgcataagcgttttgactactggggccagggaaccctggtcaccgtttcgagaggcggtggcggatcgtctgagctgactcaggaccctgctgtgtctgtggccttgggacagacagtcaggatcacatgccaaggagacagcctcagaagctattatgcaagctggtaccagcagaagccaggacaggcccctgtacttgtcatctatggtaaaaacaaccggccctcagggatcccagaccgattctctggctccagctcaggaaacacagcttccttgaccatcactggggctcaggcggaagatgaggctgactattactgtaactcctcttttccccggacttcttctgtggtattcggcggagggaccaagctgaccgtcctaggc

SEQ ID NO: 21 - protein, 100 aa, Artificial Sequence
  Amino acid sequence of the extracellular domain of CD99
DGGFDLSDALPDNENKKPTAIPKKPSAGDDFDLGDAVVDGENDDPRPPNPPKPMPNPNPNHPSSSGSFSDADLADGVSGGEGKGGSDGGGSHRKEGEEAD

SEQ ID NO: 22 - DNA, 300 bp, Artificial Sequence
  coding sequence for the extracellular domain of CD99
gatggtggtttcgatttatccgatgcccttcctgacaatgagaacaagaaacccactgcaatccccaagaaacccagtgctggggatgactttgacttaggagatgctgttgttgatggagaaaatgacgacccacgaccaccgaacccacccaaaccgatgccaaatccaaaccccaaccaccctagttcctccggtagcttttcagatgctgaccttgcggatggcgtttcaggtggagaaggaaaaggaggcagtgatggtggaggcagccacaggaaagaaggggaagaggccgac

SEQ ID NO: 23 - protein, 25 aa, Artificial Sequence
  Epitope: amino acids 50-74 of the extracellular domain of CD99
GDDFDLGDAVVDGENDDPRPPNPPK

SEQ ID NO: 24 - DNA, 22 bp, Artificial Sequence
  Primer For for scFvC7 VH
ccagccggccatggccgaggtg

SEQ ID NO: 25 - DNA, 30 bp, Artificial Sequence
  Primer Rev for scFvC7 VH
gtcaccgtgtcgagaggcggtggcggatcg

SEQ ID NO: 26 - DNA, 30 bp, Artificial Sequence
  Primer For for scFvC7 VL
cgatccgccaccgcctctcgacacggtgac

SEQ ID NO: 27 - DNA, 27 bp, Artificial Sequence
  Primer Rev for scFvC7 VL
atcgaattcctagcctaggacggtcag

SEQ ID NO: 28 - DNA, 26 bp, Artificial Sequence
  Primer For CD99BamHI
ggaacggatccgatggtggtttcgat

SEQ ID NO: 29 - DNA, 28 bp, Artificial Sequence
  Primer Rev CD99_EcoRI
ggctggaattcctagtcggcctcttccc

SEQ ID NO: 30 - DNA, 23 bp, Artificial Sequence
  Primer For AGM_CD99_BamHI
gtcgcggatccgatgatggtttc

SEQ ID NO: 31 - DNA, 28 bp, Artificial Sequence
  Primer Rev AGM_CD99_BamHI
atcacgaattcctagtccgcctcctccc

SEQ ID NO: 32 - DNA, 25 bp, Artificial Sequence
  Primer For mmCD99BamHI
ggcgcggatccgacgacttcaacct

SEQ ID NO: 33 - DNA, 29 bp, Artificial Sequence
  Primer Rev mmCD99EcoRI
accacgaattcctacaagccctggggcgt

SEQ ID NO: 34 - protein, 443 aa, Artificial Sequence
  Amino acid sequence of the entire IgG4 heavy chain
EVQLVESGGGLVRPGGSLRLSCAASGFTFSSYAMSWVRQAPGKGLEWVSAISGSGGSTYYADSVKGRFTISRDNSKNTLYLQMNSLRAEDTAVYYCAKSHKRFDYWGQGTLVTVSRASTKGPSVFPLAPCSRSTSESTAALGCLVKDYFPEPVTVSWNSGALTSGVHTFPAVLQSSGLYSLSSVVTVPSSSLGTKTYTCNVDHKPSNTKVDKRVESKYGPPCPSCPAPEFLGGPSVFLFPPKPKDTLMISRTPEVTCVVVDVSQEDPEVQFNWYVDGVEVHNAKTKPREEQFNSTYRVVSVLTVLHQDWLNGKEYKCKVSNKGLPSSIEKTISKAKGQPREPQVYTLPPSQEEMTKNQVSLTCLVKGFYPSDIAVEWESNGQPENNYKTTPPVLDSDGSFFLYSRLTVDKSRWQEGNVFSCSVMHEALHNHYTQKSLSLSLGK

SEQ ID NO: 35 - protein, 214 aa, Artificial Sequence
  Amino acid sequence of the entire IgG4 light chain
SSELTQDPAVSVALGQTVRITCQGDSLRSYYASWYQQKPGQAPVLVIYGKNNRPSGIPDRFSGSSSGNTASLTITGAQAEDEADYYCNSSFPRTSSVVFGGGTKLTVLGQPKANPTVTLFPPSSEELQANKATLVCLISDFYPGAVTVAWKADGSPVKAGVETTKPSKQSNNKYAASSYLSLTPEQWKSHRSYSCQVTHEGSTVEKTVAPTECS

SEQ ID NO: 36 - DNA, 1332 bp, Artificial Sequence
  Nucleotide sequence of the entire IgG4 heavy chain
gaagtgcagctggttgagtctggcggaggactcgttagacctggcggaagcctgagactgtcttgtgccgccagcggcttcacctttagcagctacgccatgagctgggtccgacaggctcctggcaaaggccttgaatgggtgtccgccatctctggctctggcggcagcacatattacgccgactctgtgaagggcagattcaccatcagccgggacaacagcaagaacaccctgtacctgcagatgaacagcctgagagccgaggacaccgccgtgtactactgtgccaagagccacaagagattcgactactggggccagggcaccctggtcacagtgtctagagcctctacaaagggccccagcgtgttccctctggctccttgtagcagaagcaccagcgagtctacagccgctctgggctgtctggtcaaggactactttcccgagcctgtgaccgtgtcctggaatagcggagcactgacaagcggcgtgcacacctttccagctgtgctgcaaagcagcggcctgtactctctgagcagcgtcgtgacagtgcctagcagctctctgggcaccaagacctacacctgtaatgtggaccacaagcctagcaacaccaaggtggacaagcgcgtggaatctaagtacggccctccttgtcctagctgccccgctcctgaatttctcggcggaccttccgtgttcctgtttcctccaaagcctaaggacaccctgatgatcagcagaacccctgaagtgacctgcgtggtggtggacgtgtcccaagaggatcctgaggtgcagttcaattggtacgtggacggcgtggaagtgcacaacgccaagaccaagcctagagaggaacagttcaacagcacctacagagtggtgtccgtgctgaccgtgctgcaccaggattggctgaacggcaaagagtacaagtgcaaggtgtccaacaagggcctgccaagcagcatcgagaaaaccatcagcaaggccaagggccagcctagggaaccccaggtttacacactgcctccaagccaagaggaaatgaccaagaaccaggtgtccctgacctgcctcgtgaagggcttctacccttccgatatcgccgtggaatgggagagcaatggccagccagagaacaactacaagacaacccctcctgtgctggacagcgacggctcattcttcctgtacagcagactgaccgtggacaagagcagatggcaagagggcaacgtgttcagctgcagcgtgatgcacgaggccctgcacaaccactacacccagaagtctctgagcctgagcctgggcaaatga

SEQ ID NO: 37 - DNA, 645 bp, Artificial Sequence
  Nucleotide sequence of the entire IgG4 light chain
tctagtgaactgacccaggatccagccgtgtctgtggctctgggccagacagtgcggattacctgtcagggcgatagcctgagaagctactacgccagctggtatcagcagaagcctggacaggctcccgtgctggtcatctacggcaagaacaacagacccagcggcatccccgatagattcagcggctctagctctggcaataccgccagcctgacaatcactggcgcccaggctgaagatgaggccgactactactgcaacagcagcttccccagaaccagcagcgtggtgtttggcggcggaacaaagctgacagtgctgggccagcctaaggccaatcctaccgtgacactgttccctccaagcagcgaagaactgcaggccaacaaggccacactcgtgtgcctgatcagcgacttttatcctggcgccgtgaccgtggcctggaaggctgatggatctcctgtgaaagccggcgtggaaaccaccaagcctagcaagcagagcaacaacaaatacgccgccagcagctacctgagcctgacacctgagcagtggaagtcccacagatcctacagctgccaagtgacccacgagggcagcaccgtggaaaaaacagtggcccctaccgagtgcagctga

SEQ ID NO: 38 - protein, 446 aa, Artificial Sequence
  Amino acid sequence of the entire IgG1 heavy chain
EVQLVESGGGLVRPGGSLRLSCAASGFTFSSYAMSWVRQAPGKGLEWVSAISGSGGSTYYADSVKGRFTISRDNSKNTLYLQMNSLRAEDTAVYYCAKSHKRFDYWGQGTLVTVSRASTKGPSVFPLAPSSKSTSGGTAALGCLVKDYFPEPVTVSWNSGALTSGVHTFPAVLQSSGLYSLSSVVTVPSSSLGTQTYICNVNHKPSNTKVDKKVEPKSCDKTHTCPPCPAPELLGGPSVFLFPPKPKDTLMISRTPEVTCVVVDVSHEDPEVKFNWYVDGVEVHNAKTKPREEQYNSTYRVVSVLTVLHQDWLNGKEYKCKVSNKALPAPIEKTISKAKGQPREPQVYTLPPSRDELTKNQVSLTCLVKGFYPSDIAVEWESNGQPENNYKTTPPVLDSDGSFFLYSKLTVDKSRWQQGNVFSCSVMHEALHNHYTQKSLSLSPGK

SEQ ID NO: 39 - protein, 214 aa, Artificial Sequence; identical to SEQ ID NO: 35
  Amino acid sequence of the entire IgG1 light chain

SEQ ID NO: 40 - DNA, 1338 bp, Artificial Sequence
  Nucleotide sequence of the entire IgG1 heavy chain
gaagtgcagctggttgagtctggcggaggactcgttagacctggcggaagcctgagactgtcttgtgccgccagcggcttcacctttagcagctacgccatgagctgggtccgacaggctcctggcaaaggccttgaatgggtgtccgccatctctggctctggcggcagcacatattacgccgactctgtgaagggcagattcaccatcagccgggacaacagcaagaacaccctgtacctgcagatgaacagcctgagagccgaggacaccgccgtgtactactgtgccaagagccacaagagattcgactactggggccagggcaccctggtcacagtgtctagagccagcaccaagggcccttccgtgtttccactggccccctcctctaaatccacatctggcggcaccgccgccctgggctgtctggtgaaggactacttcccagagcctgtgacagtgtcctggaactctggcgccctgacatccggcgtgcacacatttccagccgtgctgcagagctccggcctgtacagcctgtctagcgtggtgacagtgccctcctctagcctgggcacacagacctatatctgcaacgtgaatcacaagccaagcaataccaaggtggacaagaaggtggagcccaagtcctgtgataagacacacacctgccccccttgtcctgctcccgagctgctgggcggccctagcgtgttcctgtttccacccaagcctaaggacaccctgatgatctcccggacacccgaggtgacctgcgtggtggtggacgtgtctcacgaggatcctgaggtgaagttcaactggtatgtggatggcgtggaggtgcacaatgccaagaccaagcccagagaggagcagtacaactctacatatagggtggtgagcgtgctgaccgtgctgcaccaggactggctgaacggcaaggagtataagtgcaaggtgtccaataaggccctgcccgcccccatcgagaagacaatcagcaaggccaagggccagcctcgggagccacaggtgtacaccctgcctccatccagagacgagctgacaaagaaccaggtgtctctgacatgtctggtgaagggcttctatcctagcgatatcgccgtggagtgggagtccaatggccagccagagaacaattacaagaccacaccccctgtgctggactccgatggctccttctttctgtattccaagctgaccgtggataagtctcggtggcagcagggcaacgtgttcagctgttccgtgatgcacgaagccctgcataatcactatactcagaaatccctgtccctgtcacctggaaag

SEQ ID NO: 41 - DNA, 642 bp, Artificial Sequence
  Nucleotide sequence of the entire IgG1 light chain
tctagtgaactgacccaggatccagccgtgtctgtggctctgggccagacagtgcggattacctgtcagggcgatagcctgagaagctactacgccagctggtatcagcagaagcctggacaggctcccgtgctggtcatctacggcaagaacaacagacccagcggcatccccgatagattcagcggctctagctctggcaataccgccagcctgacaatcactggcgcccaggctgaagatgaggccgactactactgcaacagcagcttccccagaaccagcagcgtggtgtttggcggcggaacaaagctgacagtgctgggccagcctaaggccaatcctaccgtgacactgttccctccaagcagcgaagaactgcaggccaacaaggccacactcgtgtgcctgatcagcgacttttatcctggcgccgtgaccgtggcctggaaggctgatggatctcctgtgaaagccggcgtggaaaccaccaagcctagcaagcagagcaacaacaaatacgccgccagcagctacctgagcctgacacctgagcagtggaagtcccacagatcctacagctgccaagtgacccacgagggcagcaccgtggaaaaaacagtggcccctaccgagtgcagc

SEQ ID NO: 42 - protein, 443 aa, Artificial Sequence
  Nucleotide sequence of the entire IgG4 heavy chain mutated in S228P
EVQLVESGGGLVRPGGSLRLSCAASGFTFSSYAMSWVRQAPGKGLEWVSAISGSGGSTYYADSVKGRFTISRDNSKNTLYLQMNSLRAEDTAVYYCAKSHKRFDYWGQGTLVTVSRASTKGPSVFPLAPCSRSTSESTAALGCLVKDYFPEPVTVSWNSGALTSGVHTFPAVLQSSGLYSLSSVVTVPSSSLGTKTYTCNVDHKPSNTKVDKRVESKYGPPCPPCPAPEFLGGPSVFLFPPKPKDTLMISRTPEVTCVVVDVSQEDPEVQFNWYVDGVEVHNAKTKPREEQFNSTYRVVSVLTVLHQDWLNGKEYKCKVSNKGLPSSIEKTISKAKGQPREPQVYTLPPSQEEMTKNQVSLTCLVKGFYPSDIAVEWESNGQPENNYKTTPPVLDSDGSFFLYSRLTVDKSRWQEGNVFSCSVMHEALHNHYTQKSLSLSLGK